European Patent Application EP 4 737 484 A1, published May 6, 2026. Title: BISPECIFIC ANTIBODY TARGETING PD-L1 AND IL-1 AND USE THEREOF. Applicant: PHIL RIVERS TECHNOLOGY CO., LTD. Application CN. The sequence listing filed with the application follows.

SEQUENCE LISTING (72 sequences)

SEQ ID NO: 1 - protein, 153 aa, Homo sapiens
APVRSLNCTLRDSQQKSLVMSGPYELKALHLQGQDMEQQVVFSMSFVQGEESNDKIPVALGLKEKNLYLSCVLKDDKPTLQLESVDPKNYPKKKMEKRFVFNKIEINNKLEFESAQFPNWYISTSQAENMPVFLGGTKGGQDITDFTMQFVSS

SEQ ID NO: 2 - protein, 319 aa, Homo sapiens
LEADKCKEREEKIILVSSANEIDVRPCPLNPNEHKGTITWYKDDSKTPVSTEQASRIHQHKEKLWFVPAKVEDSGHYYCVVRNSSYCLRIKISAKFVENEPNLCYNAQAIFKQKLPVAGDGGLVCPYMEFFKNENNELPKLQWYKDCKPLLLDNIHFSGVKDRLIVMNVAEKHRGNYTCHASYTYLGKQYPITRVIEFITLEENKPTRPVIVSPANETMEVDLGSQIQLICNVTGQLSDIAYWKWNGSVIDEDDPVLGEDYYSVENPANKRRSTLITVLNISEIESRFYKHPFTCFAKNTHGIDAAYIQLIYPVTNFQK

SEQ ID NO: 3 - protein, 220 aa, Homo sapiens
FTVTVPKDLYVVEYGSNMTIECKFPVEKQLDLAALIVYWEMEDKNIIQFVHGEEDLKVQHSSYRQRARLLKDQLSLGNAALQITDVKLQDAGVYRCMISYGGADYKRITVKVNAPYNKINQRILVVDPVTSEHELTCQAEGYPKAEVIWTSSDHQVLSGKTTTTNSKREEKLFNVTSTLRINTTTNEIFYCTFRRLDPEENHTAELVIPELPLAHPPNER

SEQ ID NO: 4 - protein, 232 aa, Homo sapiens
EPKSCDKTHTCPPCPAPELLGGPSVFLFPPKPKDTLMISRTPEVTCVVVDVSHEDPEVKFNWYVDGVEVHNAKTKPREEQYNSTYRVVSVLTVLHQDWLNGKEYKCKVSNKALPAPIEKTISKAKGQPREPQVYTLPPSRDELTKNQVSLTCLVKGFYPSDIAVEWESNGQPENNYKTTPPVLDSDGSFFLYSKLTVDKSRWQQGNVFSCSVMHEALHNHYTQKSLSLSPGK

SEQ ID NO: 5 - protein, 6 aa, synthetic construct
HHHHHH

SEQ ID NO: 6 - protein, 214 aa, synthetic construct
EIVLTQSPDFQSVTPKEKVTITCRASQSIGSSLHWYQQKPDQSPKLLIKYASQSFSGVPSRFSGSGSGTDFTLTINSLEAEDAAAYYCHQSSSLPFTFGPGTKVDIKRTVAAPSVFIFPPSDEQLKSGTASVVCLLNNFYPREAKVQWKVDNALQSGNSQESVTEQDSKDSTYSLSSTLTLSKADYEKHKVYACEVTHQGLSSPVTKSFNRGEC

SEQ ID NO: 7 - protein, 448 aa, synthetic construct
QVQLVESGGGVVQPGRSLRLSCAASGFTFSVYGMNWVRQAPGKGLEWVAIIWYDGDNQYYADSVKGRFTISRDNSKNTLYLQMNGLRAEDTAVYYCARDLRTGPFDYWGQGTLVTVSSASTKGPSVFPLAPSSKSTSGGTAALGCLVKDYFPEPVTVSWNSGALTSGVHTFPAVLQSSGLYSLSSVVTVPSSSLGTQTYICNVNHKPSNTKVDKRVEPKSCDKTHTCPPCPAPELLGGPSVFLFPPKPKDTLMISRTPEVTCVVVDVSHEDPEVKFNWYVDGVEVHNAKTKPREEQYNSTYRVVSVLTVLHQDWLNGKEYKCKVSNKALPAPIEKTISKAKGQPREPQVYTLPPSREEMTKNQVSLTCLVKGFYPSDIAVEWESNGQPENNYKTTPPVLDSDGSFFLYSKLTVDKSRWQQGNVFSCSVMHEALHNHYTQKSLSLSPGK

SEQ ID NO: 8 - protein, 214 aa, synthetic construct
DIQMTQSPSSLSASVGDRVTITCRASQDVSTAVAWYQQKPGKAPKLLIYSASFLYSGVPSRFSGSGSGTDFTLTISSLQPEDFATYYCQQYLYHPATFGQGTKVEIKRTVAAPSVFIFPPSDEQLKSGTASVVCLLNNFYPREAKVQWKVDNALQSGNSQESVTEQDSKDSTYSLSSTLTLSKADYEKHKVYACEVTHQGLSSPVTKSFNRGEC

SEQ ID NO: 9 - protein, 448 aa, synthetic construct
EVQLVESGGGLVQPGGSLRLSCAASGFTFSDSWIHWVRQAPGKGLEWVAWISPYGGSTYYADSVKGRFTISADTSKNTAYLQMNSLRAEDTAVYYCARRHWPGGFDYWGQGTLVTVSSASTKGPSVFPLAPSSKSTSGGTAALGCLVKDYFPEPVTVSWNSGALTSGVHTFPAVLQSSGLYSLSSVVTVPSSSLGTQTYICNVNHKPSNTKVDKKVEPKSCDKTHTCPPCPAPELLGGPSVFLFPPKPKDTLMISRTPEVTCVVVDVSHEDPEVKFNWYVDGVEVHNAKTKPREEQYASTYRVVSVLTVLHQDWLNGKEYKCKVSNKALPAPIEKTISKAKGQPREPQVYTLPPSREEMTKNQVSLTCLVKGFYPSDIAVEWESNGQPENNYKTTPPVLDSDGSFFLYSKLTVDKSRWQQGNVFSCSVMHEALHNHYTQKSLSLSPGK

SEQ ID NO: 10 - protein, 384 aa, synthetic construct
RPSGRKSSKMQAFRIWDVNQKTFYLRNNQLVAGYLQGPNVNLEEKIDVVPIEPHALFLGIHGGKMCLSCVKSGDETRLQLEAVNITDLSENRKQDKRFAFIRSDSGPTTSFESAACPGWFLCTAMEADQPVSLTNMPDEGVMVTKFYFQEDEEPKSCDKTHTCPPCPAPELLGGPSVFLFPPKPKDTLMISRTPEVTCVVVDVSHEDPEVKFNWYVDGVEVHNAKTKPREEQYNSTYRVVSVLTVLHQDWLNGKEYKCKVSNKALPAPIEKTISKAKGQPREPQVYTLPPSRDELTKNQVSLTCLVKGFYPSDIAVEWESNGQPENNYKTTPPVLDSDGSFFLYSKLTVDKSRWQQGNVFSCSVMHEALHNHYTQKSLSLSPGK

SEQ ID NO: 11 - protein, 569 aa, Homo sapiens
MKVLLRLICFIALLISFLEADKCNEREEKIILVSSANEIDVRPCPLNPNEYKGTITWYKNDSKTPISTEQASRIHQHKKKLWFVPAKVEDSGHYYCVVRNSSYCLRIKITAKFVENEPNLCYNAEAIFKQRLPVAGDGGLVCPYMEFFKDENNELPKLLWYKDCKPLLLDNIHFSGVKDRLIVMNVAEKHRGNYTCHASYTYLGKQYPITRVIEFITLEENKPTRPVIVSPANETIEVDLGSQIQLICNVTGQLSDTAYWKWNGSFIDEDDPVLGEDYYSVENPANKRRSTLITVLNISETESRFYKHPFTCLARNTHGMDAAYVQLIYPVTKFQKHMIGICVTLTVIIMCSVFIYKIFKVDIVLWYRDSCYDFLPIKASDGKTYDAYILYPKTAGEGSTSDCDIFVFKVLPEVLEKQCGYKLFIFGRDDYVGEDIVEVINENVKKSRRLIIILVREISGFSWLGGSSEEQIAMYNALVQDGIKVVLLELEKIQDYEKMPESIKFIKRKHGVIRWSGDFTQGPQSAKTRFWKNVRYHMPVQRRSPSSKHQLPSPATKEKLQREAHVPLG

SEQ ID NO: 12 - protein, 290 aa, Homo sapiens
MRIFAVFIFMTYWHLLNAFTVTVPKDLYVVEYGSNMTIECKFPVEKQLDLAALIVYWEMEDKNIIQFVHGEEDLKVQHSSYRQRARLLKDQLSLGNAALQITDVKLQDAGVYRCMISYGGADYKRITVKVNAPYNKINQRILVVDPVTSEHELTCQAEGYPKAEVIWTSSDHQVLSGKTTTTNSKREEKLFNVTSTLRINTTTNEIFYCTFRRLDPEENHTAELVIPELPLAHPPNERTHLVILGAILLCLGVALTFIFRLRKGRMMDVKKCGIQDTNSKKQSDTHLEET

SEQ ID NO: 13 - protein, 288 aa, Homo sapiens
MQIPQAPWPVVWAVLQLGWRPGWFLDSPDRPWNPPTFSPALLVVTEGDNATFTCSFSNTSESFVLNWYRMSPSNQTDKLAAFPEDRSQPGQDCRFRVTQLPNGRDFHMSVVRARRNDSGTYLCGAISLAPKAQIKESLRAELRVTERRAEVPTAHPSPSPRPAGQFQTLVVGVVGGLLGSLVLLVWVLAVICSRAARGTIGARRTGQPLKEDPSAVPVFSVDYGELDFQWREKTPEPPVPCVPEQTEYATIVFPSGMGTSSPARRGSADGPRSAQPLRPEDGHCSWPL

SEQ ID NO: 14 - protein, 152 aa, synthetic construct
RPSGRKSSKMQAFRIWDVNQKTFYLRNNQLVAGYLQGPNVNLEEKIDVVPIEPHALFLGIHGGKMCLSCVKSGDETRLQLEAVNITDLSENRKQDKRFAFIRSDSGPTTSFESAACPGWFLCTAMEADQPVSLTNMPDEGVMVTKFYFQEDE

SEQ ID NO: 15 - protein, 118 aa, synthetic construct [sequence omitted]

SEQ ID NO: 16 - protein, 107 aa, synthetic construct [sequence omitted]

SEQ ID NO: 17 - protein, 118 aa, synthetic construct [sequence omitted]

SEQ ID NO: 18 - protein, 107 aa, synthetic construct [sequence omitted]

SEQ ID NO: 19 - protein, 16 aa, synthetic construct
GGGGSGGGGSGGGGSG

SEQ ID NO: 20 - protein, 21 aa, synthetic construct
GGGGSGGGGSGGGGSGGGGSG

SEQ ID NO: 21 - protein, 15 aa, synthetic construct
GGGGSGGGGSGGGGS

SEQ ID NO: 22 - protein, 20 aa, synthetic construct
GGGGSGGGGSGGGGSGGGGS

SEQ ID NO: 23 - protein, 12 aa, synthetic construct
TVAAPSVFIFPP

SEQ ID NO: 24 - protein, 13 aa, synthetic construct
ASTKGPSVFPLAP

SEQ ID NO: 25 - protein, 448 aa, synthetic construct
EVQLVESGGGLVQPGGSLRLSCAASGFTFSDSWIHWVRQAPGKGLEWVAWISPYGGSTYYADSVKGRFTISADTSKNTAYLQMNSLRAEDTAVYYCARRHWPGGFDYWGQGTLVTVSSASTKGPSVFPLAPSSKSTSGGTAALGCLVKDYFPEPVTVSWNSGALTSGVHTFPAVLQSSGLYSLSSVVTVPSSSLGTQTYICNVNHKPSNTKVDKKVEPKSCDKTHTCPPCPAPELLGGPSVFLFPPKPKDTLMISRTPEVTCVVVDVSHEDPEVKFNWYVDGVEVHNAKTKPREEQYNSTYRVVSVLTVLHQDWLNGKEYKCKVSNKALPAPIEKTISKAKGQPREPQVYTLPPSRDELTKNQVSLTCLVKGFYPSDIAVEWESNGQPENNYKTTPPVLDSDGSFFLYSKLTVDKSRWQQGNVFSCSVMHEALHNHYTQKSLSLSPGK

SEQ ID NO: 26 - protein, 387 aa, synthetic construct
RPSGRKSSKMQAFRIWDVNQKTFYLRNNQLVAGYLQGPNVNLEEKIDVVPIEPHALFLGIHGGKMCLSCVKSGDETRLQLEAVNITDLSENRKQDKRFAFIRSDSGPTTSFESAACPGWFLCTAMEADQPVSLTNMPDEGVMVTKFYFQEDEGGGGSGGGGSGGGGSGGGGSGDIQMTQSPSSLSASVGDRVTITCRASQDVSTAVAWYQQKPGKAPKLLIYSASFLYSGVPSRFSGSGSGTDFTLTISSLQPEDFATYYCQQYLYHPATFGQGTKVEIKRTVAAPSVFIFPPSDEQLKSGTASVVCLLNNFYPREAKVQWKVDNALQSGNSQESVTEQDSKDSTYSLSSTLTLSKADYEKHKVYACEVTHQGLSSPVTKSFNRGEC

SEQ ID NO: 27 - protein, 621 aa, synthetic construct
RPSGRKSSKMQAFRIWDVNQKTFYLRNNQLVAGYLQGPNVNLEEKIDVVPIEPHALFLGIHGGKMCLSCVKSGDETRLQLEAVNITDLSENRKQDKRFAFIRSDSGPTTSFESAACPGWFLCTAMEADQPVSLTNMPDEGVMVTKFYFQEDEGGGGSGGGGSGGGGSGGGGSGEVQLVESGGGLVQPGGSLRLSCAASGFTFSDSWIHWVRQAPGKGLEWVAWISPYGGSTYYADSVKGRFTISADTSKNTAYLQMNSLRAEDTAVYYCARRHWPGGFDYWGQGTLVTVSSASTKGPSVFPLAPSSKSTSGGTAALGCLVKDYFPEPVTVSWNSGALTSGVHTFPAVLQSSGLYSLSSVVTVPSSSLGTQTYICNVNHKPSNTKVDKKVEPKSCDKTHTCPPCPAPELLGGPSVFLFPPKPKDTLMISRTPEVTCVVVDVSHEDPEVKFNWYVDGVEVHNAKTKPREEQYASTYRVVSVLTVLHQDWLNGKEYKCKVSNKALPAPIEKTISKAKGQPREPQVYTLPPSREEMTKNQVSLTCLVKGFYPSDIAVEWESNGQPENNYKTTPPVLDSDGSFFLYSKLTVDKSRWQQGNVFSCSVMHEALHNHYTQKSLSLSPGK

SEQ ID NO: 28 - protein, 214 aa, synthetic construct; identical to SEQ ID NO: 8

SEQ ID NO: 29 - protein, 616 aa, synthetic construct
RPSGRKSSKMQAFRIWDVNQKTFYLRNNQLVAGYLQGPNVNLEEKIDVVPIEPHALFLGIHGGKMCLSCVKSGDETRLQLEAVNITDLSENRKQDKRFAFIRSDSGPTTSFESAACPGWFLCTAMEADQPVSLTNMPDEGVMVTKFYFQEDEGGGGSGGGGSGGGGSGEVQLVESGGGLVQPGGSLRLSCAASGFTFSDSWIHWVRQAPGKGLEWVAWISPYGGSTYYADSVKGRFTISADTSKNTAYLQMNSLRAEDTAVYYCARRHWPGGFDYWGQGTLVTVSSASTKGPSVFPLAPSSKSTSGGTAALGCLVKDYFPEPVTVSWNSGALTSGVHTFPAVLQSSGLYSLSSVVTVPSSSLGTQTYICNVNHKPSNTKVDKKVEPKSCDKTHTCPPCPAPELLGGPSVFLFPPKPKDTLMISRTPEVTCVVVDVSHEDPEVKFNWYVDGVEVHNAKTKPREEQYASTYRVVSVLTVLHQDWLNGKEYKCKVSNKALPAPIEKTISKAKGQPREPQVYTLPPSREEMTKNQVSLTCLVKGFYPSDIAVEWESNGQPENNYKTTPPVLDSDGSFFLYSKLTVDKSRWQQGNVFSCSVMHEALHNHYTQKSLSLSPGK

SEQ ID NO: 30 - protein, 387 aa, synthetic construct
DIQMTQSPSSLSASVGDRVTITCRASQDVSTAVAWYQQKPGKAPKLLIYSASFLYSGVPSRFSGSGSGTDFTLTISSLQPEDFATYYCQQYLYHPATFGQGTKVEIKRTVAAPSVFIFPPSDEQLKSGTASVVCLLNNFYPREAKVQWKVDNALQSGNSQESVTEQDSKDSTYSLSSTLTLSKADYEKHKVYACEVTHQGLSSPVTKSFNRGECGGGGSGGGGSGGGGSGGGGSGRPSGRKSSKMQAFRIWDVNQKTFYLRNNQLVAGYLQGPNVNLEEKIDVVPIEPHALFLGIHGGKMCLSCVKSGDETRLQLEAVNITDLSENRKQDKRFAFIRSDSGPTTSFESAACPGWFLCTAMEADQPVSLTNMPDEGVMVTKFYFQEDE

SEQ ID NO: 31 - protein, 621 aa, synthetic construct
EVQLVESGGGLVQPGGSLRLSCAASGFTFSDSWIHWVRQAPGKGLEWVAWISPYGGSTYYADSVKGRFTISADTSKNTAYLQMNSLRAEDTAVYYCARRHWPGGFDYWGQGTLVTVSSASTKGPSVFPLAPSSKSTSGGTAALGCLVKDYFPEPVTVSWNSGALTSGVHTFPAVLQSSGLYSLSSVVTVPSSSLGTQTYICNVNHKPSNTKVDKKVEPKSCDKTHTCPPCPAPELLGGPSVFLFPPKPKDTLMISRTPEVTCVVVDVSHEDPEVKFNWYVDGVEVHNAKTKPREEQYNSTYRVVSVLTVLHQDWLNGKEYKCKVSNKALPAPIEKTISKAKGQPREPQVYTLPPSRDELTKNQVSLTCLVKGFYPSDIAVEWESNGQPENNYKTTPPVLDSDGSFFLYSKLTVDKSRWQQGNVFSCSVMHEALHNHYTQKSLSLSPGKGGGGSGGGGSGGGGSGGGGSGRPSGRKSSKMQAFRIWDVNQKTFYLRNNQLVAGYLQGPNVNLEEKIDVVPIEPHALFLGIHGGKMCLSCVKSGDETRLQLEAVNITDLSENRKQDKRFAFIRSDSGPTTSFESAACPGWFLCTAMEADQPVSLTNMPDEGVMVTKFYFQEDE

SEQ ID NO: 32 - protein, 616 aa, synthetic construct
EVQLVESGGGLVQPGGSLRLSCAASGFTFSDSWIHWVRQAPGKGLEWVAWISPYGGSTYYADSVKGRFTISADTSKNTAYLQMNSLRAEDTAVYYCARRHWPGGFDYWGQGTLVTVSSASTKGPSVFPLAPSSKSTSGGTAALGCLVKDYFPEPVTVSWNSGALTSGVHTFPAVLQSSGLYSLSSVVTVPSSSLGTQTYICNVNHKPSNTKVDKKVEPKSCDKTHTCPPCPAPELLGGPSVFLFPPKPKDTLMISRTPEVTCVVVDVSHEDPEVKFNWYVDGVEVHNAKTKPREEQYNSTYRVVSVLTVLHQDWLNGKEYKCKVSNKALPAPIEKTISKAKGQPREPQVYTLPPSRDELTKNQVSLTCLVKGFYPSDIAVEWESNGQPENNYKTTPPVLDSDGSFFLYSKLTVDKSRWQQGNVFSCSVMHEALHNHYTQKSLSLSPGKGGGGSGGGGSGGGGSGRPSGRKSSKMQAFRIWDVNQKTFYLRNNQLVAGYLQGPNVNLEEKIDVVPIEPHALFLGIHGGKMCLSCVKSGDETRLQLEAVNITDLSENRKQDKRFAFIRSDSGPTTSFESAACPGWFLCTAMEADQPVSLTNMPDEGVMVTKFYFQEDE

SEQ ID NO: 33 - protein, 448 aa, synthetic construct
EVQLVESGGGLVQPGGSLRLSCAASGFTFSDSWIHWVRQAPGKGLEWVAWISPYGGSTYYADSVKGRFTISADTSKNTAYLQMNSLRAEDTAVYYCARRHWPGGFDYWGQGTLVTVSSASTKGPSVFPLAPSSKSTSGGTAALGCLVKDYFPEPVTVSWNSGALTSGVHTFPAVLQSSGLYSLSSVVTVPSSSLGTQTYICNVNHKPSNTKVDKKVEPKSCDKTHTCPPCPAPELLGGPSVFLFPPKPKDTLMISRTPEVTCVVVDVSHEDPEVKFNWYVDGVEVHNAKTKPREEQYNSTYRVVSVLTVLHQDWLNGKEYKCKVSNKALPAPIEKTISKAKGQPREPQVYTLPPCRDELTKNQVSLWCLVKGFYPSDIAVEWESNGQPENNYKTTPPVLDSDGSFFLYSKLTVDKSRWQQGNVFSCSVMHEALHNHYTQKSLSLSPGK

SEQ ID NO: 34 - protein, 621 aa, synthetic construct
RPSGRKSSKMQAFRIWDVNQKTFYLRNNQLVAGYLQGPNVNLEEKIDVVPIEPHALFLGIHGGKMCLSCVKSGDETRLQLEAVNITDLSENRKQDKRFAFIRSDSGPTTSFESAACPGWFLCTAMEADQPVSLTNMPDEGVMVTKFYFQEDEGGGGSGGGGSGGGGSGGGGSGEVQLVESGGGLVQPGGSLRLSCAASGFTFSDSWIHWVRQAPGKGLEWVAWISPYGGSTYYADSVKGRFTISADTSKNTAYLQMNSLRAEDTAVYYCARRHWPGGFDYWGQGTLVTVSSASTKGPSVFPLAPSSKSTSGGTAALGCLVKDYFPEPVTVSWNSGALTSGVHTFPAVLQSSGLYSLSSVVTVPSSSLGTQTYICNVNHKPSNTKVDKKVEPKSCDKTHTCPPCPAPELLGGPSVFLFPPKPKDTLMISRTPEVTCVVVDVSHEDPEVKFNWYVDGVEVHNAKTKPREEQYNSTYRVVSVLTVLHQDWLNGKEYKCKVSNKALPAPIEKTISKAKGQPREPQVCTLPPSRDELTKNQVSLSCAVKGFYPSDIAVEWESNGQPENNYKTTPPVLDSDGSFFLVSKLTVDKSRWQQGNVFSCSVMHEALHNHYTQKSLSLSPGK

SEQ ID NO: 35 - protein, 452 aa, synthetic construct
EVQLVESGGGLVQPGGSLRLSCAASGFTFSDSWIHWVRQAPGKGLEWVAWISPYGGSTYYADSVKGRFTISADTSKNTAYLQMNSLRAEDTAVYYCARRHWPGGFDYWGQGTLVTVSSASVAAPSVFIFPPSDEQLKSGTASVVCLLNNFYPREAKVQWKVDNALQSGNSQESVTEQDSKDSTYSLSSTLTLSKADYEKHKVYACEVTHQGLSSPVTKSFNRGECDKTHTCPPCPAPELLGGPSVFLFPPKPKDTLMISRTPEVTCVVVDVSHEDPEVKFNWYVDGVEVHNAKTKPREEQYNSTYRVVSVLTVLHQDWLNGKEYKCKVSNKALPAPIEKTISKAKGQPREPQVCTLPPSRDELTKNQVSLSCAVKGFYPSDIAVEWESNGQPENNYKTTPPVLDSDGSFFLVSKLTVDKSRWQQGNVFSCSVMHEALHNHYTQKSLSLSPGK

SEQ ID NO: 36 - protein, 385 aa, synthetic construct
RPSGRKSSKMQAFRIWDVNQKTFYLRNNQLVAGYLQGPNVNLEEKIDVVPIEPHALFLGIHGGKMCLSCVKSGDETRLQLEAVNITDLSENRKQDKRFAFIRSDSGPTTSFESAACPGWFLCTAMEADQPVSLTNMPDEGVMVTKFYFQEDEGGGGSGGGGSGGGGSGGGGSGDIQMTQSPSSLSASVGDRVTITCRASQDVSTAVAWYQQKPGKAPKLLIYSASFLYSGVPSRFSGSGSGTDFTLTISSLQPEDFATYYCQQYLYHPATFGQGTKVEIKSSASTKGPSVFPLAPSSKSTSGGTAALGCLVKDYFPEPVTVSWNSGALTSGVHTFPAVLQSSGLYSLSSVVTVPSSSLGTQTYICNVNHKPSNTKVDKKVEPKSC

SEQ ID NO: 37 - protein, 439 aa, synthetic construct
DIQMTQSPSSLSASVGDRVTITCRASQDVSTAVAWYQQKPGKAPKLLIYSASFLYSGVPSRFSGSGSGTDFTLTISSLQPEDFATYYCQQYLYHPATFGQGTKVEIKSSASTKGPSVFPLAPSSKSTSGGTAALGCLVKDYFPEPVTVSWNSGALTSGVHTFPAVLQSSGLYSLSSVVTVPSSSLGTQTYICNVNHKPSNTKVDKKVEPKSCDKTHTCPPCPAPELLGGPSVFLFPPKPKDTLMISRTPEVTCVVVDVSHEDPEVKFNWYVDGVEVHNAKTKPREEQYNSTYRVVSVLTVLHQDWLNGKEYKCKVSNKALPAPIEKTISKAKGQPREPQVCTLPPSRDELTKNQVSLSCAVKGFYPSDIAVEWESNGQPENNYKTTPPVLDSDGSFFLVSKLTVDKSRWQQGNVFSCSVMHEALHNHYTQKSLSLSPGK

SEQ ID NO: 38 - protein, 398 aa, synthetic construct
EVQLVESGGGLVQPGGSLRLSCAASGFTFSDSWIHWVRQAPGKGLEWVAWISPYGGSTYYADSVKGRFTISADTSKNTAYLQMNSLRAEDTAVYYCARRHWPGGFDYWGQGTLVTVSSASVAAPSVFIFPPSDEQLKSGTASVVCLLNNFYPREAKVQWKVDNALQSGNSQESVTEQDSKDSTYSLSSTLTLSKADYEKHKVYACEVTHQGLSSPVTKSFNRGECGGGGSGGGGSGGGGSGGGGSGRPSGRKSSKMQAFRIWDVNQKTFYLRNNQLVAGYLQGPNVNLEEKIDVVPIEPHALFLGIHGGKMCLSCVKSGDETRLQLEAVNITDLSENRKQDKRFAFIRSDSGPTTSFESAACPGWFLCTAMEADQPVSLTNMPDEGVMVTKFYFQEDE

SEQ ID NO: 39 - protein, 621 aa, synthetic construct
EVQLVESGGGLVQPGGSLRLSCAASGFTFSDSWIHWVRQAPGKGLEWVAWISPYGGSTYYADSVKGRFTISADTSKNTAYLQMNSLRAEDTAVYYCARRHWPGGFDYWGQGTLVTVSSASTKGPSVFPLAPSSKSTSGGTAALGCLVKDYFPEPVTVSWNSGALTSGVHTFPAVLQSSGLYSLSSVVTVPSSSLGTQTYICNVNHKPSNTKVDKKVEPKSCDKTHTCPPCPAPELLGGPSVFLFPPKPKDTLMISRTPEVTCVVVDVSHEDPEVKFNWYVDGVEVHNAKTKPREEQYNSTYRVVSVLTVLHQDWLNGKEYKCKVSNKALPAPIEKTISKAKGQPREPQVCTLPPSRDELTKNQVSLSCAVKGFYPSDIAVEWESNGQPENNYKTTPPVLDSDGSFFLVSKLTVDKSRWQQGNVFSCSVMHEALHNHYTQKSLSLSPGKGGGGSGGGGSGGGGSGGGGSGRPSGRKSSKMQAFRIWDVNQKTFYLRNNQLVAGYLQGPNVNLEEKIDVVPIEPHALFLGIHGGKMCLSCVKSGDETRLQLEAVNITDLSENRKQDKRFAFIRSDSGPTTSFESAACPGWFLCTAMEADQPVSLTNMPDEGVMVTKFYFQEDE

SEQ ID NO: 40 - protein, 608 aa, synthetic construct
NTAYLQMNSLRAEDTAVYYCARRHWPGGFDYWGQGTLVTVSSASTKGPSVFPLAPSSKSTSGGTAALGCLVKDYFPEPVTVSWNSGALTSGVHTFPAVLQSSGLYSLSSVVTVPSSSLGTQTYICNVNHKPSNTKVDKKVEPKSCDKTHTCPPCPAPELLGGPSVFLFPPKPKDTLMISRTPEVTCVVVDVSHEDPEVKFNWYVDGVEVHNAKTKPREEQYNSTYRVVSVLTVLHQDWLNGKEYKCKVSNKALPAPIEKTISKAKGQPREPQVYTLPPCRDELTKNQVSLWCLVKGFYPSDIAVEWESNGQPENNYKTTPPVLDSDGSFFLYSKLTVDKSRWQQGNVFSCSVMHEALHNHYTQKSLSLSPGKGGGGSGGGGSGGGGSEVQLVESGGGLVQPGGSLRLSCAASGFTFSDSWIHWVRQAPGKGLEWVAWISPYGGSTYYADSVKGRFTISADTSKNTAYLQMNSLRAEDTAVYYCARRHWPGGFDYWGQGTLVTVSSASTKGPSVFPLAPSSKSTSGGTAALGCLVKDYFPEPVTVSWNSGALTSGVHTFPAVLQSSGLYSLSSVVTVPSSSLGTQTYICNVNHKPSNTKVDKKVEPKSC

SEQ ID NO: 41 - protein, 581 aa, synthetic construct
QVQLVESGGGVVQPGRSLRLSCAASGFTFSVYGMNWVRQAPGKGLEWVAIIWYDGDNQYYADSVKGRFTISRDNSKNTLYLQMNGLRAEDTAVYYCARDLRTGPFDYWGQGTLVTVSSGGGGSGGGGSGGGGSEVQLVESGGGLVQPGGSLRLSCAASGFTFSDSWIHWVRQAPGKGLEWVAWISPYGGSTYYADSVKGRFTISADTSKNTAYLQMNSLRAEDTAVYYCARRHWPGGFDYWGQGTLVTVSSASTKGPSVFPLAPSSKSTSGGTAALGCLVKDYFPEPVTVSWNSGALTSGVHTFPAVLQSSGLYSLSSVVTVPSSSLGTQTYICNVNHKPSNTKVDKKVEPKSCDKTHTCPPCPAPELLGGPSVFLFPPKPKDTLMISRTPEVTCVVVDVSHEDPEVKFNWYVDGVEVHNAKTKPREEQYASTYRVVSVLTVLHQDWLNGKEYKCKVSNKALPAPIEKTISKAKGQPREPQVYTLPPSREEMTKNQVSLTCLVKGFYPSDIAVEWESNGQPENNYKTTPPVLDSDGSFFLYSKLTVDKSRWQQGNVFSCSVMHEALHNHYTQKSLSLSPGK

SEQ ID NO: 42 - protein, 336 aa, synthetic construct
EIVLTQSPDFQSVTPKEKVTITCRASQSIGSSLHWYQQKPDQSPKLLIKYASQSFSGVPSRFSGSGSGTDFTLTINSLEAEDAAAYYCHQSSSLPFTFGPGTKVDIKGGGGSGGGGSGGGGSDIQMTQSPSSLSASVGDRVTITCRASQDVSTAVAWYQQKPGKAPKLLIYSASFLYSGVPSRFSGSGSGTDFTLTISSLQPEDFATYYCQQYLYHPATFGQGTKVEIKRTVAAPSVFIFPPSDEQLKSGTASVVCLLNNFYPREAKVQWKVDNALQSGNSQESVTEQDSKDSTYSLSSTLTLSKADYEKHKVYACEVTHQGLSSPVTKSFNRGEC

SEQ ID NO: 43 - protein, 579 aa, synthetic construct
QVQLVESGGGVVQPGRSLRLSCAASGFTFSVYGMNWVRQAPGKGLEWVAIIWYDGDNQYYADSVKGRFTISRDNSKNTLYLQMNGLRAEDTAVYYCARDLRTGPFDYWGQGTLVTVSSASTKGPSVFPLAPEVQLVESGGGLVQPGGSLRLSCAASGFTFSDSWIHWVRQAPGKGLEWVAWISPYGGSTYYADSVKGRFTISADTSKNTAYLQMNSLRAEDTAVYYCARRHWPGGFDYWGQGTLVTVSSASTKGPSVFPLAPSSKSTSGGTAALGCLVKDYFPEPVTVSWNSGALTSGVHTFPAVLQSSGLYSLSSVVTVPSSSLGTQTYICNVNHKPSNTKVDKKVEPKSCDKTHTCPPCPAPELLGGPSVFLFPPKPKDTLMISRTPEVTCVVVDVSHEDPEVKFNWYVDGVEVHNAKTKPREEQYASTYRVVSVLTVLHQDWLNGKEYKCKVSNKALPAPIEKTISKAKGQPREPQVYTLPPSREEMTKNQVSLTCLVKGFYPSDIAVEWESNGQPENNYKTTPPVLDSDGSFFLYSKLTVDKSRWQQGNVFSCSVMHEALHNHYTQKSLSLSPGK

SEQ ID NO: 44 - protein, 333 aa, synthetic construct
EIVLTQSPDFQSVTPKEKVTITCRASQSIGSSLHWYQQKPDQSPKLLIKYASQSFSGVPSRFSGSGSGTDFTLTINSLEAEDAAAYYCHQSSSLPFTFGPGTKVDIKTVAAPSVFIFPPDIQMTQSPSSLSASVGDRVTITCRASQDVSTAVAWYQQKPGKAPKLLIYSASFLYSGVPSRFSGSGSGTDFTLTISSLQPEDFATYYCQQYLYHPATFGQGTKVEIKRTVAAPSVFIFPPSDEQLKSGTASVVCLLNNFYPREAKVQWKVDNALQSGNSQESVTEQDSKDSTYSLSSTLTLSKADYEKHKVYACEVTHQGLSSPVTKSFNRGEC

SEQ ID NO: 45 - protein, 581 aa, synthetic construct
EVQLVESGGGLVQPGGSLRLSCAASGFTFSDSWIHWVRQAPGKGLEWVAWISPYGGSTYYADSVKGRFTISADTSKNTAYLQMNSLRAEDTAVYYCARRHWPGGFDYWGQGTLVTVSSGGGGSGGGGSGGGGSQVQLVESGGGVVQPGRSLRLSCAASGFTFSVYGMNWVRQAPGKGLEWVAIIWYDGDNQYYADSVKGRFTISRDNSKNTLYLQMNGLRAEDTAVYYCARDLRTGPFDYWGQGTLVTVSSASTKGPSVFPLAPSSKSTSGGTAALGCLVKDYFPEPVTVSWNSGALTSGVHTFPAVLQSSGLYSLSSVVTVPSSSLGTQTYICNVNHKPSNTKVDKRVEPKSCDKTHTCPPCPAPELLGGPSVFLFPPKPKDTLMISRTPEVTCVVVDVSHEDPEVKFNWYVDGVEVHNAKTKPREEQYNSTYRVVSVLTVLHQDWLNGKEYKCKVSNKALPAPIEKTISKAKGQPREPQVYTLPPSREEMTKNQVSLTCLVKGFYPSDIAVEWESNGQPENNYKTTPPVLDSDGSFFLYSKLTVDKSRWQQGNVFSCSVMHEALHNHYTQKSLSLSPGK

SEQ ID NO: 46 - protein, 336 aa, synthetic construct
DIQMTQSPSSLSASVGDRVTITCRASQDVSTAVAWYQQKPGKAPKLLIYSASFLYSGVPSRFSGSGSGTDFTLTISSLQPEDFATYYCQQYLYHPATFGQGTKVEIKGGGGSGGGGSGGGGSEIVLTQSPDFQSVTPKEKVTITCRASQSIGSSLHWYQQKPDQSPKLLIKYASQSFSGVPSRFSGSGSGTDFTLTINSLEAEDAAAYYCHQSSSLPFTFGPGTKVDIKRTVAAPSVFIFPPSDEQLKSGTASVVCLLNNFYPREAKVQWKVDNALQSGNSQESVTEQDSKDSTYSLSSTLTLSKADYEKHKVYACEVTHQGLSSPVTKSFNRGEC

SEQ ID NO: 47 - protein, 703 aa, synthetic construct
EVQLVESGGGLVQPGGSLRLSCAASGFTFSDSWIHWVRQAPGKGLEWVAWISPYGGSTYYADSVKGRFTISADTSKNTAYLQMNSLRAEDTAVYYCARRHWPGGFDYWGQGTLVTVSSASTKGPSVFPLAPSSKSTSGGTAALGCLVKDYFPEPVTVSWNSGALTSGVHTFPAVLQSSGLYSLSSVVTVPSSSLGTQTYICNVNHKPSNTKVDKKVEPKSCDKTHTCPPCPAPELLGGPSVFLFPPKPKDTLMISRTPEVTCVVVDVSHEDPEVKFNWYVDGVEVHNAKTKPREEQYASTYRVVSVLTVLHQDWLNGKEYKCKVSNKALPAPIEKTISKAKGQPREPQVYTLPPSREEMTKNQVSLTCLVKGFYPSDIAVEWESNGQPENNYKTTPPVLDSDGSFFLYSKLTVDKSRWQQGNVFSCSVMHEALHNHYTQKSLSLSPGKGGGGSGGGGSGGGGSQVQLVESGGGVVQPGRSLRLSCAASGFTFSVYGMNWVRQAPGKGLEWVAIIWYDGDNQYYADSVKGRFTISRDNSKNTLYLQMNGLRAEDTAVYYCARDLRTGPFDYWGQGTLVTVSSGGGGSGGGGSGGGGSEIVLTQSPDFQSVTPKEKVTITCRASQSIGSSLHWYQQKPDQSPKLLIKYASQSFSGVPSRFSGSGSGTDFTLTINSLEAEDAAAYYCHQSSSLPFTFGPGTKVDIK

SEQ ID NO: 48 - protein, 441 aa, synthetic construct
EIVLTQSPDFQSVTPKEKVTITCRASQSIGSSLHWYQQKPDQSPKLLIKYASQSFSGVPSRFSGSGSGTDFTLTINSLEAEDAAAYYCHQSSSLPFTFGPGTKVDIKRTVAAPSVFIFPPSDEQLKSGTASVVCLLNNFYPREAKVQWKVDNALQSGNSQESVTEQDSKDSTYSLSSTLTLSKADYEKHKVYACEVTHQGLSSPVTKSFNRGECDKTHTCPPCPAPELLGGPSVFLFPPKPKDTLMISRTPEVTCVVVDVSHEDPEVKFNWYVDGVEVHNAKTKPREEQYNSTYRVVSVLTVLHQDWLNGKEYKCKVSNKALPAPIEKTISKAKGQPREPQVCTLPPSRDELTKNQVSLSCAVKGFYPSDIAVEWESNGQPENNYKTTPPVLDSDGSFFLVSKLTVDKSRWQQGNVFSCSVMHEALHNHYTQKSLSLSPGK

SEQ ID NO: 49 - protein, 221 aa, synthetic construct
QVQLVESGGGVVQPGRSLRLSCAASGFTFSVYGMNWVRQAPGKGLEWVAIIWYDGDNQYYADSVKGRFTISRDNSKNTLYLQMNGLRAEDTAVYYCARDLRTGPFDYWGQGTLVTVSSASTKGPSVFPLAPSSKSTSGGTAALGCLVKDYFPEPVTVSWNSGALTSGVHTFPAVLQSSGLYSLSSVVTVPSSSLGTQTYICNVNHKPSNTKVDKKVEPKSC

SEQ ID NO: 50 - protein, 452 aa, synthetic construct
QVQLVESGGGVVQPGRSLRLSCAASGFTFSVYGMNWVRQAPGKGLEWVAIIWYDGDNQYYADSVKGRFTISRDNSKNTLYLQMNGLRAEDTAVYYCARDLRTGPFDYWGQGTLVTVSSASVAAPSVFIFPPSDEQLKSGTASVVCLLNNFYPREAKVQWKVDNALQSGNSQESVTEQDSKDSTYSLSSTLTLSKADYEKHKVYACEVTHQGLSSPVTKSFNRGECDKTHTCPPCPAPELLGGPSVFLFPPKPKDTLMISRTPEVTCVVVDVSHEDPEVKFNWYVDGVEVHNAKTKPREEQYNSTYRVVSVLTVLHQDWLNGKEYKCKVSNKALPAPIEKTISKAKGQPREPQVCTLPPSRDELTKNQVSLSCAVKGFYPSDIAVEWESNGQPENNYKTTPPVLDSDGSFFLVSKLTVDKSRWQQGNVFSCSVMHEALHNHYTQKSLSLSPGK

SEQ ID NO: 51 - protein, 212 aa, synthetic construct
EIVLTQSPDFQSVTPKEKVTITCRASQSIGSSLHWYQQKPDQSPKLLIKYASQSFSGVPSRFSGSGSGTDFTLTINSLEAEDAAAYYCHQSSSLPFTFGPGTKVDIKSSASTKGPSVFPLAPSSKSTSGGTAALGCLVKDYFPEPVTVSWNSGALTSGVHTFPAVLQSSGLYSLSSVVTVPSSSLGTQTYICNVNHKPSNTKVDKKVEPKSC

SEQ ID NO: 52 - protein, 439 aa, synthetic construct
EIVLTQSPDFQSVTPKEKVTITCRASQSIGSSLHWYQQKPDQSPKLLIKYASQSFSGVPSRFSGSGSGTDFTLTINSLEAEDAAAYYCHQSSSLPFTFGPGTKVDIKSSASTKGPSVFPLAPSSKSTSGGTAALGCLVKDYFPEPVTVSWNSGALTSGVHTFPAVLQSSGLYSLSSVVTVPSSSLGTQTYICNVNHKPSNTKVDKKVEPKSCDKTHTCPPCPAPELLGGPSVFLFPPKPKDTLMISRTPEVTCVVVDVSHEDPEVKFNWYVDGVEVHNAKTKPREEQYNSTYRVVSVLTVLHQDWLNGKEYKCKVSNKALPAPIEKTISKAKGQPREPQVCTLPPSRDELTKNQVSLSCAVKGFYPSDIAVEWESNGQPENNYKTTPPVLDSDGSFFLVSKLTVDKSRWQQGNVFSCSVMHEALHNHYTQKSLSLSPGK

SEQ ID NO: 53 - protein, 225 aa, synthetic construct
QVQLVESGGGVVQPGRSLRLSCAASGFTFSVYGMNWVRQAPGKGLEWVAIIWYDGDNQYYADSVKGRFTISRDNSKNTLYLQMNGLRAEDTAVYYCARDLRTGPFDYWGQGTLVTVSSASVAAPSVFIFPPSDEQLKSGTASVVCLLNNFYPREAKVQWKVDNALQSGNSQESVTEQDSKDSTYSLSSTLTLSKADYEKHKVYACEVTHQGLSSPVTKSFNRGEC

SEQ ID NO: 54 - protein, 703 aa, synthetic construct
EVQLVESGGGLVQPGGSLRLSCAASGFTFSDSWIHWVRQAPGKGLEWVAWISPYGGSTYYADSVKGRFTISADTSKNTAYLQMNSLRAEDTAVYYCARRHWPGGFDYWGQGTLVTVSSASTKGPSVFPLAPSSKSTSGGTAALGCLVKDYFPEPVTVSWNSGALTSGVHTFPAVLQSSGLYSLSSVVTVPSSSLGTQTYICNVNHKPSNTKVDKKVEPKSCDKTHTCPPCPAPELLGGPSVFLFPPKPKDTLMISRTPEVTCVVVDVSHEDPEVKFNWYVDGVEVHNAKTKPREEQYNSTYRVVSVLTVLHQDWLNGKEYKCKVSNKALPAPIEKTISKAKGQPREPQVYTLPPCRDELTKNQVSLWCLVKGFYPSDIAVEWESNGQPENNYKTTPPVLDSDGSFFLYSKLTVDKSRWQQGNVFSCSVMHEALHNHYTQKSLSLSPGKGGGGSGGGGSGGGGSQVQLVESGGGVVQPGRSLRLSCAASGFTFSVYGMNWVRQAPGKGLEWVAIIWYDGDNQYYADSVKGRFTISRDNSKNTLYLQMNGLRAEDTAVYYCARDLRTGPFDYWGQGTLVTVSSGGGGSGGGGSGGGGSEIVLTQSPDFQSVTPKEKVTITCRASQSIGSSLHWYQQKPDQSPKLLIKYASQSFSGVPSRFSGSGSGTDFTLTINSLEAEDAAAYYCHQSSSLPFTFGPGTKVDIK

SEQ ID NO: 55 - protein, 448 aa, synthetic construct
EVQLVESGGGLVQPGGSLRLSCAASGFTFSDSWIHWVRQAPGKGLEWVAWISPYGGSTYYADSVKGRFTISADTSKNTAYLQMNSLRAEDTAVYYCARRHWPGGFDYWGQGTLVTVSSASTKGPSVFPLAPSSKSTSGGTAALGCLVKDYFPEPVTVSWNSGALTSGVHTFPAVLQSSGLYSLSSVVTVPSSSLGTQTYICNVNHKPSNTKVDKKVEPKSCDKTHTCPPCPAPELLGGPSVFLFPPKPKDTLMISRTPEVTCVVVDVSHEDPEVKFNWYVDGVEVHNAKTKPREEQYNSTYRVVSVLTVLHQDWLNGKEYKCKVSNKALPAPIEKTISKAKGQPREPQVCTLPPSRDELTKNQVSLSCAVKGFYPSDIAVEWESNGQPENNYKTTPPVLDSDGSFFLVSKLTVDKSRWQQGNVFSCSVMHEALHNHYTQKSLSLSPGK

SEQ ID NO: 56 - protein, 482 aa, synthetic construct
QVQLVESGGGVVQPGRSLRLSCAASGFTFSVYGMNWVRQAPGKGLEWVAIIWYDGDNQYYADSVKGRFTISRDNSKNTLYLQMNGLRAEDTAVYYCARDLRTGPFDYWGQGTLVTVSSGGGGSGGGGSGGGGSEIVLTQSPDFQSVTPKEKVTITCRASQSIGSSLHWYQQKPDQSPKLLIKYASQSFSGVPSRFSGSGSGTDFTLTINSLEAEDAAAYYCHQSSSLPFTFGPGTKVDIKGGGGSGGGGSGGGGSDKTHTCPPCPAPELLGGPSVFLFPPKPKDTLMISRTPEVTCVVVDVSHEDPEVKFNWYVDGVEVHNAKTKPREEQYNSTYRVVSVLTVLHQDWLNGKEYKCKVSNKALPAPIEKTISKAKGQPREPQVCTLPPSRDELTKNQVSLSCAVKGFYPSDIAVEWESNGQPENNYKTTPPVLDSDGSFFLVSKLTVDKSRWQQGNVFSCSVMHEALHNHYTQKSLSLSPGK

SEQ ID NO: 57 - protein, 703 aa, synthetic construct
EVQLVESGGGLVQPGGSLRLSCAASGFTFSDSWIHWVRQAPGKGLEWVAWISPYGGSTYYADSVKGRFTISADTSKNTAYLQMNSLRAEDTAVYYCARRHWPGGFDYWGQGTLVTVSSASTKGPSVFPLAPSSKSTSGGTAALGCLVKDYFPEPVTVSWNSGALTSGVHTFPAVLQSSGLYSLSSVVTVPSSSLGTQTYICNVNHKPSNTKVDKKVEPKSCDKTHTCPPCPAPELLGGPSVFLFPPKPKDTLMISRTPEVTCVVVDVSHEDPEVKFNWYVDGVEVHNAKTKPREEQYNSTYRVVSVLTVLHQDWLNGKEYKCKVSNKALPAPIEKTISKAKGQPREPQVCTLPPSRDELTKNQVSLSCAVKGFYPSDIAVEWESNGQPENNYKTTPPVLDSDGSFFLVSKLTVDKSRWQQGNVFSCSVMHEALHNHYTQKSLSLSPGKGGGGSGGGGSGGGGSQVQLVESGGGVVQPGRSLRLSCAASGFTFSVYGMNWVRQAPGKGLEWVAIIWYDGDNQYYADSVKGRFTISRDNSKNTLYLQMNGLRAEDTAVYYCARDLRTGPFDYWGQGTLVTVSSGGGGSGGGGSGGGGSEIVLTQSPDFQSVTPKEKVTITCRASQSIGSSLHWYQQKPDQSPKLLIKYASQSFSGVPSRFSGSGSGTDFTLTINSLEAEDAAAYYCHQSSSLPFTFGPGTKVDIK

SEQ ID NO: 58 - protein, 448 aa, synthetic construct
EVQLVESGGGLVQPGGSLRLSCAASGFTFSDSWIHWVRQAPGKGLEWVAWISPYGGSTYYADSVKGRFTISADTSKNTAYLQMNSLRAEDTAVYYCARRHWPGGFDYWGQGTLVTVSSASTKGPSVFPLAPSSKSTSGGTAALGCLVKDYFPEPVTVSWNSGALTSGVHTFPAVLQSSGLYSLSSVVTVPSSSLGTQTYICNVNHKPSNTKVDKRVEPKSCDKTHTCPPCPAPELLGGPSVFLFPPKPKDTLMISRTPEVTCVVVDVSHEDPEVKFNWYVDGVEVHNAKTKPREEQYNSTYRVVSVLTVLHQDWLNGKEYKCKVSNKALPAPIEKTISKAKGQPREPQVYTLPPSREEMTKNQVSLTCLVKGFYPSDIAVEWESNGQPENNYKTTPPVLDSDGSFLLYSKLTVDKSRWQQGNVFSCSVMHEALHNHYTQKSLSLSPGK

SEQ ID NO: 59 - protein, 452 aa, synthetic construct
QVQLVESGGGVVQPGRSLRLSCAASGFTFSVYGMNWVRQAPGKGLEWVAIIWYDGDNQYYADSVKGRFTISRDNSKNTLYLQMNGLRAEDTAVYYCARDLRTGPFDYWGQGTLVTVSSASVAAPSVFIFPPSDEQLKSGTASVVCLLNNFYPREAKVQWKVDNALQSGNSQESVTEQDSKDSTYSLSSTLTLSKADYEKHKVYACEVTHQGLSSPVTKSFNRGECDKTHTCPPCPAPELLGGPSVFLFPPKPKDTLMISRTPEVTCVVVDVSHEDPEVKFNWYVDGVEVHNAKTKPREEQYNSTYRVVSVLTVLHQDWLNGKEYKCKVSNKALPAPIEKTISKAKGQPREPQVYTLPPSREEMTKNQVSLTCLVKGFYPSDIAVEWESNGQPENNYKTTPPVLDSDGSFFLYSRLTVDKSRWQQGNVFSCSVMHEALHNHYTQKSLSLSPGK

SEQ ID NO: 60 - protein, 212 aa, synthetic construct
EIVLTQSPDFQSVTPKEKVTITCRASQSIGSSLHWYQQKPDQSPKLLIKYASQSFSGVPSRFSGSGSGTDFTLTINSLEAEDAAAYYCHQSSSLPFTFGPGTKVDIKSSASTKGPSVFPLAPSSKSTSGGTAALGCLVKDYFPEPVTVSWNSGALTSGVHTFPAVLQSSGLYSLSSVVTVPSSSLGTQTYICNVNHKPSNTKVDKRVEPKSC

SEQ ID NO: 61 - protein, 713 aa, synthetic construct
EVQLVESGGGLVQPGGSLRLSCAASGFTFSDSWIHWVRQAPGKGLEWVAWISPYGGSTYYADSVKGRFTISADTSKNTAYLQMNSLRAEDTAVYYCARRHWPGGFDYWGQGTLVTVSSASTKGPSVFPLAPSSKSTSGGTAALGCLVKDYFPEPVTVSWNSGALTSGVHTFPAVLQSSGLYSLSSVVTVPSSSLGTQTYICNVNHKPSNTKVDKKVEPKSCDKTHTCPPCPAPELLGGPSVFLFPPKPKDTLMISRTPEVTCVVVDVSHEDPEVKFNWYVDGVEVHNAKTKPREEQYASTYRVVSVLTVLHQDWLNGKEYKCKVSNKALPAPIEKTISKAKGQPREPQVYTLPPSREEMTKNQVSLTCLVKGFYPSDIAVEWESNGQPENNYKTTPPVLDSDGSFFLYSKLTVDKSRWQQGNVFSCSVMHEALHNHYTQKSLSLSPGKGGGGSGGGGSGGGGSGGGGSQVQLVESGGGVVQPGRSLRLSCAASGFTFSVYGMNWVRQAPGKGLEWVAIIWYDGDNQYYADSVKGRFTISRDNSKNTLYLQMNGLRAEDTAVYYCARDLRTGPFDYWGQGTLVTVSSGGGGSGGGGSGGGGSGGGGSEIVLTQSPDFQSVTPKEKVTITCRASQSIGSSLHWYQQKPDQSPKLLIKYASQSFSGVPSRFSGSGSGTDFTLTINSLEAEDAAAYYCHQSSSLPFTFGPGTKVDIK

SEQ ID NO: 62 - protein, 713 aa, synthetic construct
QVQLVESGGGVVQPGRSLRLSCAASGFTFSVYGMNWVRQAPGKGLEWVAIIWYDGDNQYYADSVKGRFTISRDNSKNTLYLQMNGLRAEDTAVYYCARDLRTGPFDYWGQGTLVTVSSASTKGPSVFPLAPSSKSTSGGTAALGCLVKDYFPEPVTVSWNSGALTSGVHTFPAVLQSSGLYSLSSVVTVPSSSLGTQTYICNVNHKPSNTKVDKRVEPKSCDKTHTCPPCPAPELLGGPSVFLFPPKPKDTLMISRTPEVTCVVVDVSHEDPEVKFNWYVDGVEVHNAKTKPREEQYNSTYRVVSVLTVLHQDWLNGKEYKCKVSNKALPAPIEKTISKAKGQPREPQVYTLPPSREEMTKNQVSLTCLVKGFYPSDIAVEWESNGQPENNYKTTPPVLDSDGSFFLYSKLTVDKSRWQQGNVFSCSVMHEALHNHYTQKSLSLSPGKGGGGSGGGGSGGGGSGGGGSEVQLVESGGGLVQPGGSLRLSCAASGFTFSDSWIHWVRQAPGKCLEWVAWISPYGGSTYYADSVKGRFTISADTSKNTAYLQMNSLRAEDTAVYYCARRHWPGGFDYWGQGTLVTVSSGGGGSGGGGSGGGGSGGGGSDIQMTQSPSSLSASVGDRVTITCRASQDVSTAVAWYQQKPGKAPKLLIYSASFLYSGVPSRFSGSGSGTDFTLTISSLQPEDFATYYCQQYLYHPATFGCGTKVEIK

SEQ ID NO: 63 - protein, 214 aa, synthetic construct; identical to SEQ ID NO: 6

SEQ ID NO: 64 - protein, 225 aa, synthetic construct
QVQLVESGGGVVQPGRSLRLSCAASGFTFSVYGMNWVRQAPGKGLEWVAIIWYDGDNQYYADSVKGRFTISRDNSKNTLYLQMNGLRAEDTAVYYCARDLRTGPFDYWGQGTLVTVSSEIVLTQSPDFQSVTPKEKVTITCRASQSIGSSLHWYQQKPDQSPKLLIKYASQSFSGVPSRFSGSGSGTDFTLTINSLEAEDAAAYYCHQSSSLPFTFGPGTKVDIK

SEQ ID NO: 65 - protein, 225 aa, synthetic construct
EVQLVESGGGLVQPGGSLRLSCAASGFTFSDSWIHWVRQAPGKGLEWVAWISPYGGSTYYADSVKGRFTISADTSKNTAYLQMNSLRAEDTAVYYCARRHWPGGFDYWGQGTLVTVSSDIQMTQSPSSLSASVGDRVTITCRASQDVSTAVAWYQQKPGKAPKLLIYSASFLYSGVPSRFSGSGSGTDFTLTISSLQPEDFATYYCQQYLYHPATFGQGTKVEIK

SEQ ID NO: 66 - protein, 384 aa, synthetic construct
RPSGRKSSKMQAFRIWDVNQKTFYLRNNQLVAGYLQGPNVNLEEKIDVVPIEPHALFLGIHGGKMCLSCVKSGDETRLQLEAVNITDLSENRKQDKRFAFIRSDSGPTTSFESAACPGWFLCTAMEADQPVSLTNMPDEGVMVTKFYFQEDEEPKSSDKTHTCPPCPAPELLGGPSVFLFPPKPKDTLMISRTPEVTCVVVDVSHEDPEVKFNWYVDGVEVHNAKTKPREEQYASTYRVVSVLTVLHQDWLNGKEYKCKVSNKALPAPIEKTISKAKGQPREPQVYTLPPSRDELTKNQVSLTCLVKGFYPSDIAVEWESNGQPENNYKTTPPVLDSDGSFFLYSKLTVDKSRWQQGNVFSCSVMHEALHNHYTQKSLSLSPGK

SEQ ID NO: 67 - protein, 232 aa, Homo sapiens
EPKSSDKTHTCPPCPAPELLGGPSVFLFPPKPKDTLMISRTPEVTCVVVDVSHEDPEVKFNWYVDGVEVHNAKTKPREEQYASTYRVVSVLTVLHQDWLNGKEYKCKVSNKALPAPIEKTISKAKGQPREPQVYTLPPSRDELTKNQVSLTCLVKGFYPSDIAVEWESNGQPENNYKTTPPVLDSDGSFFLYSKLTVDKSRWQQGNVFSCSVMHEALHNHYTQKSLSLSPGK

SEQ ID NO: 68 - protein, 330 aa, Homo sapiens
ASTKGPSVFPLAPSSKSTSGGTAALGCLVKDYFPEPVTVSWNSGALTSGVHTFPAVLQSSGLYSLSSVVTVPSSSLGTQTYICNVNHKPSNTKVDKRVEPKSCDKTHTCPPCPAPELLGGPSVFLFPPKPKDTLMISRTPEVTCVVVDVSHEDPEVKFNWYVDGVEVHNAKTKPREEQYASTYRVVSVLTVLHQDWLNGKEYKCKVSNKALPAPIEKTISKAKGQPREPQVYTLPPSREEMTKNQVSLTCLVKGFYPSDIAVEWESNGQPENNYKTTPPVLDSDGSFFLYSKLTVDKSRWQQGNVFSCSVMHEALHNHYTQKSLSLSPGK

SEQ ID NO: 69 - protein, 448 aa, synthetic construct; identical to SEQ ID NO: 9

SEQ ID NO: 70 - protein, 616 aa, synthetic construct
EVQLVESGGGLVQPGGSLRLSCAASGFTFSDSWIHWVRQAPGKGLEWVAWISPYGGSTYYADSVKGRFTISADTSKNTAYLQMNSLRAEDTAVYYCARRHWPGGFDYWGQGTLVTVSSASTKGPSVFPLAPSSKSTSGGTAALGCLVKDYFPEPVTVSWNSGALTSGVHTFPAVLQSSGLYSLSSVVTVPSSSLGTQTYICNVNHKPSNTKVDKKVEPKSCDKTHTCPPCPAPELLGGPSVFLFPPKPKDTLMISRTPEVTCVVVDVSHEDPEVKFNWYVDGVEVHNAKTKPREEQYASTYRVVSVLTVLHQDWLNGKEYKCKVSNKALPAPIEKTISKAKGQPREPQVYTLPPSREEMTKNQVSLTCLVKGFYPSDIAVEWESNGQPENNYKTTPPVLDSDGSFFLYSKLTVDKSRWQQGNVFSCSVMHEALHNHYTQKSLSLSPGKGGGGSGGGGSGGGGSGRPSGRKSSKMQAFRIWDVNQKTFYLRNNQLVAGYLQGPNVNLEEKIDVVPIEPHALFLGIHGGKMCLSCVKSGDETRLQLEAVNITDLSENRKQDKRFAFIRSDSGPTTSFESAACPGWFLCTAMEADQPVSLTNMPDEGVMVTKFYFQEDE

SEQ ID NO: 71 - protein, 581 aa, synthetic construct
EVQLVESGGGLVQPGGSLRLSCAASGFTFSDSWIHWVRQAPGKGLEWVAWISPYGGSTYYADSVKGRFTISADTSKNTAYLQMNSLRAEDTAVYYCARRHWPGGFDYWGQGTLVTVSSGGGGSGGGGSGGGGSQVQLVESGGGVVQPGRSLRLSCAASGFTFSVYGMNWVRQAPGKGLEWVAIIWYDGDNQYYADSVKGRFTISRDNSKNTLYLQMNGLRAEDTAVYYCARDLRTGPFDYWGQGTLVTVSSASTKGPSVFPLAPSSKSTSGGTAALGCLVKDYFPEPVTVSWNSGALTSGVHTFPAVLQSSGLYSLSSVVTVPSSSLGTQTYICNVNHKPSNTKVDKRVEPKSCDKTHTCPPCPAPELLGGPSVFLFPPKPKDTLMISRTPEVTCVVVDVSHEDPEVKFNWYVDGVEVHNAKTKPREEQYASTYRVVSVLTVLHQDWLNGKEYKCKVSNKALPAPIEKTISKAKGQPREPQVYTLPPSREEMTKNQVSLTCLVKGFYPSDIAVEWESNGQPENNYKTTPPVLDSDGSFFLYSKLTVDKSRWQQGNVFSCSVMHEALHNHYTQKSLSLSPGK

SEQ ID NO: 72 - protein, 713 aa, synthetic construct
QVQLVESGGGVVQPGRSLRLSCAASGFTFSVYGMNWVRQAPGKGLEWVAIIWYDGDNQYYADSVKGRFTISRDNSKNTLYLQMNGLRAEDTAVYYCARDLRTGPFDYWGQGTLVTVSSASTKGPSVFPLAPSSKSTSGGTAALGCLVKDYFPEPVTVSWNSGALTSGVHTFPAVLQSSGLYSLSSVVTVPSSSLGTQTYICNVNHKPSNTKVDKRVEPKSCDKTHTCPPCPAPELLGGPSVFLFPPKPKDTLMISRTPEVTCVVVDVSHEDPEVKFNWYVDGVEVHNAKTKPREEQYASTYRVVSVLTVLHQDWLNGKEYKCKVSNKALPAPIEKTISKAKGQPREPQVYTLPPSREEMTKNQVSLTCLVKGFYPSDIAVEWESNGQPENNYKTTPPVLDSDGSFFLYSKLTVDKSRWQQGNVFSCSVMHEALHNHYTQKSLSLSPGKGGGGSGGGGSGGGGSGGGGSEVQLVESGGGLVQPGGSLRLSCAASGFTFSDSWIHWVRQAPGKCLEWVAWISPYGGSTYYADSVKGRFTISADTSKNTAYLQMNSLRAEDTAVYYCARRHWPGGFDYWGQGTLVTVSSGGGGSGGGGSGGGGSGGGGSDIQMTQSPSSLSASVGDRVTITCRASQDVSTAVAWYQQKPGKAPKLLIYSASFLYSGVPSRFSGSGSGTDFTLTISSLQPEDFATYYCQQYLYHPATFGCGTKVEIK